European Patent Application EP 4 378 951 A1, published June 5, 2024. Title: GENERAL AFFINITY EPITOPE POLYPEPTIDE FOR HUMAN RHINOVIRUS, AND ANTIBODY AND USES THEREOF. Applicant: BEIJING WANTAI BIOLOGICAL PHARMACY ENTERPRISE CO., LTD. Application CN. The sequence listing filed with the application follows.

SEQUENCE LISTING (52 sequences)

SEQ ID NO: 1 - protein, 13 aa, synthetic construct
  source 1..13: note = Amino acid sequence of polypeptide 2C01
YSLPPDPKYFDGY

SEQ ID NO: 2 - protein, 9 aa, synthetic construct
  source 1..9: note = Amino acid sequence of polypeptide 2C02
CNAAKGLEW

SEQ ID NO: 3 - protein, 8 aa, synthetic construct
  source 1..8: note = Amino acid sequence of polypeptide 2C03
FCQMVSTT

SEQ ID NO: 4 - protein, 183 aa, synthetic construct
  source 1..183: note = Amino acid sequence of HBcAg
MDIDPYKEFGASVELLSFLPSDFFPSIRDLLDTASALYREALESPEHCSPHHTALRQAILCWGELMNLATWVGSNLEDPASRELVVSYVNVNMGLKIRQLLWFHISCLTFGRETVLEYLVSFGVWIRTPPAYRPQNAPILSTLPETTVVRRRCRSPRRRTPSPRRRRSQSPRRRRSQSRESQC

SEQ ID NO: 5 - protein, 183 aa, synthetic construct
  source 1..183: note = Amino acid sequence of C149-2C (aa 151-163)(C149-2C01)
MDIDPYKEFGASVELLSFLPSDFFPSIRDLLDTASALYREALESPEHCSPHHTALRQAILCWGELMNLATWVGSNLEDGGGGSGGGGTGSYSLPPDPKYFDGYEFGGGGSGGGGSRELVVSYVNVNMGLKIRQLLWFHISCLTLGRETVLEYLVSFGVWIRTPPAYRPQNAPILSTLPETTVV

SEQ ID NO: 6 - protein, 179 aa, synthetic construct
  source 1..179: note = Amino acid sequence of C149-2C (aa 12-20) (C149-2C02)
MDIDPYKEFGASVELLSFLPSDFFPSIRDLLDTASALYREALESPEHCSPHHTALRQAILCWGELMNLATWVGSNLEDGGGGSGGGGTGSCNAAKGLEWEFGGGGSGGGGSRELVVSYVNVNMGLKIRQLLWFHISCLTLGRETVLEYLVSFGVWIRTPPAYRPQNAPILSTLPETTVV

SEQ ID NO: 7 - protein, 178 aa, synthetic construct
  source 1..178: note = Amino acid sequence of C149-2C (aa 186-193)(C149-2C03)
MDIDPYKEFGASVELLSFLPSDFFPSIRDLLDTASALYREALESPEHCSPHHTALRQAILCWGELMNLATWVGSNLEDGGGGSGGGGTGSFCQMVSTTEFGGGGSGGGGSRELVVSYVNVNMGLKIRQLLWFHISCLTLGRETVLEYLVSFGVWIRTPPAYRPQNAPILSTLPETTVV

SEQ ID NO: 8 - protein, 24 aa, synthetic construct
  source 1..24: note = Amino acid sequence of linker
GGGGSGGGGTGSFEFGGGGSGGGG

SEQ ID NO: 9 - protein, 326 aa, synthetic construct
  source 1..326: note = Amino acid sequence of human rhinovirus (W10(HRV-C15)) non-structural protein 2C
SDSWLRKFTECCNAAKGLEWISIKIGKFIDWLKGKLVPAVQRKRDTLDRCKKISLLEEQVNGFSSASSEAQQQLIVEVDTLKKGLDELAPLYASENKRVTKIQKDLKQLSAYLKNHRHEPVCLLLHGNPGCGKSLVTTIIARGLTQEAQVYSLPPDPKYFDGYDQQQVVILDDLGQNPDGKDLSTFCQMVSTTDFIVPMASLEDKGKSFTSQYVLASTNLDTLSPPTVTIPEAIKRRFFLDADLITTSKFRNTTGLLDVAKALQPCTGCPKPAHYKTCCPLLCGKAVVVQDRKTKANFSVNTIVEQLRHENATRKKVKHNLDAIFQ

SEQ ID NO: 10 - DNA, 45 bp, synthetic construct
  source 1..45: mol_type = other DNA; note = Nucleotide sequence of primer 1 for 2C (aa 151-163)
gatcctactcactaccacctgatcccaaatatttcgatggttatg

SEQ ID NO: 11 - DNA, 45 bp, synthetic construct
  source 1..45: mol_type = other DNA; note = Nucleotide sequence of primer 2 for 2C (aa 151-163)
aattcataaccatcgaaatatttgggatcaggtggtagtgagtag

SEQ ID NO: 12 - DNA, 33 bp, synthetic construct
  source 1..33: mol_type = other DNA; note = Nucleotide sequence of primer 1 for 2C (aa 12-20)
gatcctgcaatgcagcaaaaggacttgaatggg

SEQ ID NO: 13 - DNA, 33 bp, synthetic construct
  source 1..33: mol_type = other DNA; note = Nucleotide sequence of primer2 for 2C (aa 12-20)
aattcccattcaagtccttttgctgcattgcag

SEQ ID NO: 14 - DNA, 30 bp, synthetic construct
  source 1..30: mol_type = other DNA; note = Nucleotide sequence of primer1 for 2C (aa 186-193)
gatccttctgtcagatggtatcaacaacag

SEQ ID NO: 15 - DNA, 30 bp, synthetic construct
  source 1..30: mol_type = other DNA; note = Nucleotide sequence of primer2 for 2C (aa 186-193)
aattctgttgttgataccatctgacagaag

SEQ ID NO: 16 - DNA, 39 bp, synthetic construct
  source 1..39: mol_type = other DNA; note = Nucleotide sequence of primer MVkF-G1
actagtcgacatgaagttgcctgttaggctgttggtgct

SEQ ID NO: 17 - DNA, 30 bp, synthetic construct
  source 1..30: mol_type = other DNA; note = Nucleotide sequence of primer MVkR-M13
cccaagcttactggatggtgggaagatgga

SEQ ID NO: 18 - DNA, 339 bp, synthetic construct
  source 1..339: mol_type = other DNA; note = Nucleotide sequence encoding 9A5 light chain variable region (VL)
gatgttgtgatgacccagactccactcaccttgtcggttaccattggacaaccagcctccatctcttgcaagtcaagtcagagcctcttagatagtgatggaaagacatatttgaattggttgttacagaggccaggccagtctccaaagcgcctaatctatctggtgtctaaactggactctggagtccctgacaggttcactggcagtggatcagggacagatttcacactgaaaatcagcagagtggaggctgaggatttgggagtttattattgctggcaaggtacacatcttccgcacacgttcggaggggggaccaagctggaaacaaaacgg

SEQ ID NO: 19 - protein, 113 aa, synthetic construct
  source 1..113: note = Amino acid sequence of 9A5 light chain variable region (VL)
DVVMTQTPLTLSVTIGQPASISCKSSQSLLDSDGKTYLNWLLQRPGQSPKRLIYLVSKLDSGVPDRFTGSGSGTDFTLKISRVEAEDLGVYYCWQGTHLPHTFGGGTKLETKR

SEQ ID NO: 20 - DNA, 39 bp, synthetic construct
  source 1..39: mol_type = other DNA; note = Nucleotide sequence of primer MVhF-C1
actagtcgacatggactccaggctcaatttagttttcct

SEQ ID NO: 21 - DNA, 34 bp, synthetic construct
  source 1..34: mol_type = other DNA; note = Nucleotide sequence of primer MVhR-M13
cccaagcttccagggrccarkggataracgrtgg

SEQ ID NO: 22 - DNA, 351 bp, synthetic construct
  source 1..351: mol_type = other DNA; note = Nucleotide sequence encoding 9A5 heavy chain variable region (VH)
gaggtgcagctggtggagtctgggggagacttagtgaagcctggagggtccctgaaactctcctgtgcagcctctggattcactttcagtatctatggcatgtcttgggttcgccagactccagacaagagactggagtgggtcgcaaccattagtagtgctggtatttacacctactatccagacagtgtgaaggggcgattcaccatctccagagacaatgccaagaacaccctgtacctgcaaatgagcagtctgaagtctgaggacacagccatgtattactgtgcaagacacggctacgggttgttcgatgtctggggcgcagggaccacggtcaccgtctcctca

SEQ ID NO: 23 - protein, 117 aa, synthetic construct
  source 1..117: note = Amino acid sequence of 9A5 heavy chain variable region (VH)
EVQLVESGGDLVKPGGSLKLSCAASGFTFSIYGMSWVRQTPDKRLEWVATISSAGIYTYYPDSVKGRFTISRDNAKNTLYLQMSSLKSEDTAMYYCARHGYGLFDVWGAGTTVTVSS

SEQ ID NO: 24 - protein, 11 aa, synthetic construct
  source 1..11: note = Amino acid sequence of VL CDR1
QSLLDSDGKTY

SEQ ID NO: 25 - skipped

SEQ ID NO: 26 - protein, 9 aa, synthetic construct
  source 1..9: note = Amino acid sequence of VL CDR3
WQGTHLPHT

SEQ ID NO: 27 - protein, 8 aa, synthetic construct
  source 1..8: note = Amino acid sequence of VH CDR1
GFTFSIYG

SEQ ID NO: 28 - protein, 8 aa, synthetic construct
  source 1..8: note = Amino acid sequence of VH CDR2
ISSAGIYT

SEQ ID NO: 29 - protein, 10 aa, synthetic construct
  source 1..10: note = Amino acid sequence of VH CDR3
ARHGYGLFDV

SEQ ID NO: 30 - protein, 13 aa, synthetic construct
  source 1..13: note = Amino acid sequence of rhinovirus non-structural protein 2C aa 151-163 (2C04)
YSLPPDPKHFDGY

SEQ ID NO: 31 - protein, 13 aa, synthetic construct
  source 1..13: note = Amino acid sequence of rhinovirus non-structural protein 2C aa 151-163 (2C05)
YSLPPAPKYFDGY

SEQ ID NO: 32 - protein, 13 aa, synthetic construct
  source 1..13: note = Amino acid sequence of rhinovirus non-structural protein 2Caa 151-163 (2C06)
YSLPPSPKYFDGY

SEQ ID NO: 33 - protein, 13 aa, synthetic construct
  source 1..13: note = Amino acid sequence of rhinovirus non-structural protein 2C aa 151-163 (2C07)
YSLPPNPKHFDGY

SEQ ID NO: 34 - protein, 13 aa, synthetic construct
  source 1..13: note = Amino acid sequence of rhinovirus non-structural protein 2C aa 151-163 (2C08)
YSLPPNPKYFDGY

SEQ ID NO: 35 - protein, 17 aa, synthetic construct
  source 1..17: note = Amino acid sequence of rhinovirus non-structural protein 2C aa 149-165 (2C09)
QVYSLPPDPKYFDGYDQ

SEQ ID NO: 36 - protein, 21 aa, synthetic construct
  source 1..21: note = Amino acid sequence of rhinovirus non-structural protein 2C aa 147-167 (2C10)
EAQVYSLPPDPKYFDGYDQQQ

SEQ ID NO: 37 - protein, 25 aa, synthetic construct
  source 1..25: note = Amino acid sequence of rhinovirus non-structural protein 2C aa 145-169 (2C11)
TQEAQVYSLPPDPKYFDGYDQQQVV

SEQ ID NO: 38 - DNA, 57 bp, synthetic construct
  source 1..57: mol_type = other DNA; note = Nucleotide sequence of primer1 for 2C (aa 149-165)
gatcccaggtatactcactaccacctgatcccaaatatttcgatggttatgaccaag

SEQ ID NO: 39 - DNA, 57 bp, synthetic construct
  source 1..57: mol_type = other DNA; note = Nucleotide sequence of primer 2 for 2C (aa 149-165)
aattcttggtcataaccatcgaaatatttgggatcaggtggtagtgagtatacctgg

SEQ ID NO: 40 - DNA, 69 bp, synthetic construct
  source 1..69: mol_type = other DNA; note = Nucleotide sequence of primer 1 for 2C (aa 147-167)
gatccgaggcacaggtatactcactaccacctgatcccaaatatttcgatggttatgaccaacagcagg

SEQ ID NO: 41 - DNA, 69 bp, synthetic construct
  source 1..69: mol_type = other DNA; note = Nucleotide sequence of primer 2 for 2C (aa 147-167)
aattcctgctgttggtcataaccatcgaaatatttgggatcaggtggtagtgagtatacctgtgcctcg

SEQ ID NO: 42 - DNA, 82 bp, synthetic construct
  source 1..82: mol_type = other DNA; note = Nucleotide sequence of primer 1 for 2C (aa 145-169)
gatccacccaggaggcacaggtatactcactaccacctgatcccaaatatttcgatggttatgaccaacagcaggttgtcgg

SEQ ID NO: 43 - DNA, 81 bp, synthetic construct
  source 1..81: mol_type = other DNA; note = Nucleotide sequence of primer 2 for 2C (aa 145-169)
aattcgacaacctgctgttggtcataaccatcgaaatatttgggatcaggtggtagtgagtatacctgtgcctcctgggtg

SEQ ID NO: 44 - protein, 183 aa, synthetic construct
  source 1..183: note = Amino acid sequence of C149-2C (aa 151-163)(C149-2C04)
MDIDPYKEFGASVELLSFLPSDFFPSIRDLLDTASALYREALESPEHCSPHHTALRQAILCWGELMNLATWVGSNLEDGGGGSGGGGTGSYSLPPDPKHFDGYEFGGGGSGGGGSRELVVSYVNVNMGLKIRQLLWFHISCLTLGRETVLEYLVSFGVWIRTPPAYRPQNAPILSTLPETTVV

SEQ ID NO: 45 - protein, 183 aa, synthetic construct
  source 1..183: note = Amino acid sequence of C149-2C (aa 151-163) (C149-2C05)
MDIDPYKEFGASVELLSFLPSDFFPSIRDLLDTASALYREALESPEHCSPHHTALRQAILCWGELMNLATWVGSNLEDGGGGSGGGGTGSYSLPPAPKYFDGYEFGGGGSGGGGSRELVVSYVNVNMGLKIRQLLWFHISCLTLGRETVLEYLVSFGVWIRTPPAYRPQNAPILSTLPETTVV

SEQ ID NO: 46 - protein, 183 aa, synthetic construct
  source 1..183: note = Amino acid sequence of C149-2C (aa 151-163) (C149-2C06)
MDIDPYKEFGASVELLSFLPSDFFPSIRDLLDTASALYREALESPEHCSPHHTALRQAILCWGELMNLATWVGSNLEDGGGGSGGGGTGSYSLPPSPKYFDGYEFGGGGSGGGGSRELVVSYVNVNMGLKIRQLLWFHISCLTLGRETVLEYLVSFGVWIRTPPAYRPQNAPILSTLPETTVV

SEQ ID NO: 47 - protein, 183 aa, synthetic construct
  source 1..183: note = Amino acid sequence of C149-2C (aa 151-163)(C149-2C07)
MDIDPYKEFGASVELLSFLPSDFFPSIRDLLDTASALYREALESPEHCSPHHTALRQAILCWGELMNLATWVGSNLEDGGGGSGGGGTGSYSLPPNPKHFDGYEFGGGGSGGGGSRELVVSYVNVNMGLKIRQLLWFHISCLTLGRETVLEYLVSFGVWIRTPPAYRPQNAPILSTLPETTVV

SEQ ID NO: 48 - protein, 183 aa, synthetic construct
  source 1..183: note = Amino acid sequence of C149-2C (aa 151-163) (C149-2C08)
MDIDPYKEFGASVELLSFLPSDFFPSIRDLLDTASALYREALESPEHCSPHHTALRQAILCWGELMNLATWVGSNLEDGGGGSGGGGTGSYSLPPNPKYFDGYEFGGGGSGGGGSRELVVSYVNVNMGLKIRQLLWFHISCLTLGRETVLEYLVSFGVWIRTPPAYRPQNAPILSTLPETTVV

SEQ ID NO: 49 - protein, 187 aa, synthetic construct
  source 1..187: note = Amino acid sequence of C149-2C (aa 149-165) (C149-2C09)
MDIDPYKEFGASVELLSFLPSDFFPSIRDLLDTASALYREALESPEHCSPHHTALRQAILCWGELMNLATWVGSNLEDGGGGSGGGGTGSQVYSLPPDPKYFDGYDQEFGGGGSGGGGSRELVVSYVNVNMGLKIRQLLWFHISCLTLGRETVLEYLVSFGVWIRTPPAYRPQNAPILSTLPETTVV

SEQ ID NO: 50 - protein, 191 aa, synthetic construct
  source 1..191: note = Amino acid sequence of C149-2C (aa 147-167) (C149-2C10)
MDIDPYKEFGASVELLSFLPSDFFPSIRDLLDTASALYREALESPEHCSPHHTALRQAILCWGELMNLATWVGSNLEDGGGGSGGGGTGSEAQVYSLPPDPKYFDGYDQQQEFGGGGSGGGGSRELVVSYVNVNMGLKIRQLLWFHISCLTLGRETVLEYLVSFGVWIRTPPAYRPQNAPILSTLPETTVV

SEQ ID NO: 51 - protein, 195 aa, synthetic construct
  source 1..195: note = Amino acid sequence of C149-2C (aa 145-169) (C149-2C11)
MDIDPYKEFGASVELLSFLPSDFFPSIRDLLDTASALYREALESPEHCSPHHTALRQAILCWGELMNLATWVGSNLEDGGGGSGGGGTGSTQEAQVYSLPPDPKYFDGYDQQQVVEFGGGGSGGGGSRELVVSYVNVNMGLKIRQLLWFHISCLTLGRETVLEYLVSFGVWIRTPPAYRPQNAPILSTLPETTVV

SEQ ID NO: 52 - protein, 13 aa, synthetic construct
  source 1..13: note = formula of C149-2C (aa 151-163)
  VARIANT 6: note = X is selected from: (i) amino acid residues D, A, S, N and (ii) amino acid residues that are conservatively substituted relative to (i).
  VARIANT 9: note = X is selected from: (i) amino acid residues Y, H and (ii) amino acid residues that are conservatively substituted relative to (i).
YSLPPXPKXFDGY